European Patent Application EP 4 219 517 A1, published August 2, 2023. Title: Novel Artificial Nucleic Acids, Production Method Thereof and Use. Applicant: RIKEN GENESIS CO., LTD. The sequence listing filed with the application follows.

SEQUENCE LISTING (8 sequences)

SEQ ID NO: 1 - DNA, 12 bp, Artificial Sequence
  Antisense Strand
  misc_feature (6)..(6): n is modified t
gcgttntttgct

SEQ ID NO: 2 - DNA, 12 bp, Artificial Sequence
  Antisense Strand
  misc_feature (4)..(4): n is a, c, g, or t
  misc_feature (6)..(6): n is modified t
  misc_feature (8)..(8): n is modified t
gcgntntntgct

SEQ ID NO: 3 - DNA, 12 bp, Artificial Sequence
  Antisense Strand
  misc_feature (6)..(8): n is modified t
gcgttnnntgct

SEQ ID NO: 4 - DNA, 12 bp, Artificial Sequence
  Antisense Strand
  misc_feature (4)..(9): n is modified t
gcgnnnnnngct

SEQ ID NO: 5 - DNA, 10 bp, Artificial Sequence
  Antisense Strand
  misc_feature (9)..(9): n is modified t
ttttttttnt

SEQ ID NO: 6 - DNA, 12 bp, Artificial Sequence
  Sense Strand
agcaaaaaacgc

SEQ ID NO: 7 - RNA, 12 nt, Artificial Sequence
  Sense Strand
agcaaaaaacgc

SEQ ID NO: 8 - DNA, 10 bp, Artificial Sequence
  Oligonucleotide
tttttttttt